European Patent Application EP 4 123 015 A1, published January 25, 2023. Title: Method for purifying myocardial cell. Applicant: Kyoto University TAKEDA PHARMACEUTICAL COMPANY LIMITED. The sequence listing filed with the application follows.

SEQUENCE LISTING (2 sequences)

SEQ ID NO: 1 - protein, 720 aa, Artificial Sequence
  EmGFP-coding sequence
ATGGTGAGCAAGGGCGAGGAGCTGTTCACCGGGGTGGTGCCCATCCTGGTCGAGCTGGACGGCGACGTAAACGGCCACAAGTTCAGCGTGTCCGGCGAGGGCGAGGGCGATGCCACCTACGGCAAGCTGACCCTGAAGTTCATCTGCACCACCGGCAAGCTGCCCGTGCCCTGGCCCACCCTCGTGACCACCTTCACCTACGGCGTGCAGTGCTTCGCCCGCTACCCCGACCACATGAAGCAGCACGACTTCTTCAAGTCCGCCATGCCCGAAGGCTACGTCCAGGAGCGCACCATCTTCTTCAAGGACGACGGCAACTACAAGACCCGCGCCGAGGTGAAGTTCGAGGGCGACACCCTGGTGAACCGCATCGAGCTGAAGGGCATCGACTTCAAGGAGGACGGCAACATCCTGGGGCACAAGCTGGAGTACAACTACAACAGCCACAAGGTCTATATCACCGCCGACAAGCAGAAGAACGGCATCAAGGTGAACTTCAAGACCCGCCACAACATCGAGGACGGCAGCGTGCAGCTCGCCGACCACTACCAGCAGAACACCCCCATCGGCGACGGCCCCGTGCTGCTGCCCGACAACCACTACCTGAGCACCCAGTCCGCCCTGAGCAAAGACCCCAACGAGAAGCGCGATCACATGGTCCTGCTGGAGTTCGTGACCGCCGCCGGGATCACTCTCGGCATGGACGAGCTGTACAAGTAA

SEQ ID NO: 2 - protein, 711 aa, Artificial Sequence
  mCherry-coding sequence
ATGGTGAGCAAGGGCGAGGAGGATAACATGGCCATCATCAAGGAGTTCATGCGCTTCAAGGTGCACATGGAGGGCTCCGTGAACGGCCACGAGTTCGAGATCGAGGGCGAGGGCGAGGGCCGCCCCTACGAGGGCACCCAGACCGCCAAGCTGAAGGTGACCAAGGGTGGCCCCCTGCCCTTCGCCTGGGACATCCTGTCCCCTCAGTTCATGTACGGCTCCAAGGCCTACGTGAAGCACCCCGCCGACATCCCCGACTACTTGAAGCTGTCCTTCCCCGAGGGCTTCAAGTGGGAGCGCGTGATGAACTTCGAGGACGGCGGCGTGGTGACCGTGACCCAGGACTCCTCCCTGCAGGACGGCGAGTTCATCTACAAGGTGAAGCTGCGCGGCACCAACTTCCCCTCCGACGGCCCCGTAATGCAGAAGAAGACCATGGGCTGGGAGGCCTCCTCCGAGCGGATGTACCCCGAGGACGGCGCCCTGAAGGGCGAGATCAAGCAGAGGCTGAAGCTGAAGGACGGCGGCCACTACGACGCTGAGGTCAAGACCACCTACAAGGCCAAGAAGCCCGTGCAGCTGCCCGGCGCCTACAACGTCAACATCAAGTTGGACATCACCTCCCACAACGAGGACTACACCATCGTGGAACAGTACGAACGCGCCGAGGGCCGCCACTCCACCGGCGGCATGGACGAGCTGTACAAGTAG